European Patent Specification EP 3 319 624 B1, published November 8, 2023. Title: LYSOSOMAL DEGRADATION OF LIPIDS AND PROTEINS AND METHOD OF USE THEREOF. Applicant: University of Ottawa. Application PCT/CA2016/000192. The sequence listing filed with the application follows.

SEQUENCE LISTING (20 sequences)

SEQ ID NO: 1 - protein, 186 aa, Homo Sapiens
MLALISRLLDWFRSLFWKEEMELTLVGLQYSGKTTFVNVIASGQFSEDMIPTVGFNMRKVTKGNVTIKIWDIGGQPRFRSMWERYCRGVNAIVYMIDAADREKIEASRNELHNLLDKPQLQGIPVLVLGNKRDLPNALDEKQLIEKMNLSAIQDREICCYSISCKEKDNIDITLQWLIQHSKSRRS

SEQ ID NO: 2 - protein, 875 aa, Homo Sapiens
MHDAFEPVPILEKLPLQIDCLAAWEEWLLVGTKQGHLLLYRIRKDVGCNRFEVTLEKSNKNFSKKIQQIHVVSQFKILVSLLENNIYVHDLLTFQQITTVSKAKGASLFTCDLQHTETGEEVLRMCVAVKKKLQLYFWKDREFHELQGDFSVPDVPKSMAWCENSICVGFKRDYYLIRVDGKGSIKELFPTGKQLEPLVAPLADGKVAVGQDDLTVVLNEEGICTQKCALNWTDIPVAMEHQPPYIIAVLPRYVEIRTFEPRLLVQSIELQRPRFITSGGSNIIYVASNHFVWRLIPVPMATQIQQLLQDKQFELALQLAEMKDDSDSEKQQQIHHIKNLYAFNLFCQKRFDESMQVFAKLGTDPTHVMGLYPDLLPTDYRKQLQYPNPLPVLSGAELEKAHLALIDYLTQKRSQLVKKLNDSDHQSSTSPLMEGTPTIKSKKKLLQIIDTTLLKCYLHTNVALVAPLLRLENNHCHIEESEHVLKKAHKYSELIILYEKKGLHEKALQVLVDQSKKANSPLKGHERTVQYLQHLGTENLHLIFSYSVWVLRDFPEDGLKIFTEDLPEVESLPRDRVLGFLIENFKGLAIPYLEHIIHVWEETGSRFHNCLIQLYCEKVQGLMKEYLLSFPAGKTPVPAGEEEGELGEYRQKLLMFLEISSYYDPGRLICDFPFDGLLEERALLLGRMGKHEQALFIYVHILKDTRMAEEYCHKHYDRNKDGNKDVYLSLLRMYLSPPSIHCLGPIKLELLEPKANLQAALQVLELHHSKLDTTKALNLLPANTQINDIRIFLEKVLEENAQKKRFNQVLKNLLHAEFLRVQEERILHQQVKCIITEEKVCMVCKKKIGNSAFARYPNGVVVHYFCSKEVNPADT

SEQ ID NO: 3 - protein, 854 aa, Homo Sapiens
MAEAEEQETGSLEESTDESEEEESEEEPKLKYERLSNGVTEILQKDAASCMTVHDKFLALGTHYGKVYLLDVQGNITQKFDVSPVKINQISLDESGEHMGVCSEDGKVQVFGLYSGEEFHETFDCPIKIIAVHPHFVRSSCKQFVTGGKKLLLFERSWMNRWKSAVLHEGEGNIRSVKWRGHLIAWANNMGVKIFDIISKQRITNVPRDDISLRPDMYPCSLCWKDNVTLIIGWGTSVKVCSVKERHASEMRDLPSRYVEIVSQFETEFYISGLAPLCDQLVVLSYVKEISEKTEREYCARPRLDIIQPLSETCEEISSDALTVRGFQENECRDYHLEYSEGESLFYIVSPRDVVVAKERDQDDHIDWLLEKKKYEEALMAAEISQKNIKRHKILDIGLAYINHLVERGDYDIAARKCQKILGKNAALWEYEVYKFKEIGQLKAISPYLPRGDPVLKPLIYEMILHEFLESDYEGFATLIREWPGDLYNNSVIVQAVRDHLKKDSQNKTLLKTLAELYTYDKNYGNALEIYLTLRHKDVFQLIHKHNLFSSIKDKIVLLMDFDSEKAVDMLLDNEDKISIKKVVEELEDRPELQHVYLHKLFKRDHHKGQRYHEKQISLYAEYDRPNLLPFLRDSTHCPLEKALEICQQRNFVEETVYLLSRMGNSRSALKMIMEELHDVDKAIEFAKEQDDGELWEDLILYSIDKPPFITGLLNNIGTHVDPILLIHRIKEGMEIPNLRDSLVKILQDYNLQILLREGCKKILVADSLSLLKKMHRTQMKGVLVDEENICESCLSPILPSDAAKPFSVVVFHCRHMFHKECLPMPSMNSAAQFCNICSAKNRGPGSAILEMKK

SEQ ID NO: 4 - protein, 829 aa, Homo Sapiens
MAEAEEQETGSLEESTDESEEEESEEEPKLKYERLSNGVTEILQKDAASCMTVHDKFLALGTHYGKVYLLDVQGNITQKFDVVQVFGLYSGEEFHETFDCPIKIIAVHPHFVRSSCKQFVTGGKKLLLFERSWMNRWKSAVLHEGEGNIRSVKWRGHLIAWANNMGVKIFDIISKQRITNVPRDDISLRPDMYPCSLCWKDNVTLIIGWGTSVKVCSVKERHASEMRDLPSRYVEIVSQFETEFYISGLAPLCDQLVVLSYVKEISEKTEREYCARPRLDIIQPLSETCEEISSDALTVRGFQENECRDYHLEYSEGESLFYIVSPRDVVVAKERDQDDHIDWLLEKKKYEEALMAAEISQKNIKRHKILDIGLAYINHLVERGDYDIAARKCQKILGKNAALWEYEVYKFKEIGQLKAISPYLPRGDPVLKPLIYEMILHEFLESDYEGFATLIREWPGDLYNNSVIVQAVRDHLKKDSQNKTLLKTLAELYTYDKNYGNALEIYLTLRHKDVFQLIHKHNLFSSIKDKIVLLMDFDSEKAVDMLLDNEDKISIKKVVEELEDRPELQHVYLHKLFKRDHHKGQRYHEKQISLYAEYDRPNLLPFLRDSTHCPLEKALEICQQRNFVEETVYLLSRMGNSRSALKMIMEELHDVDKAIEFAKEQDDGELWEDLILYSIDKPPFITGLLNNIGTHVDPILLIHRIKEGMEIPNLRDSLVKILQDYNLQILLREGCKKILVADSLSLLKKMHRTQMKGVLVDEENICESCLSPILPSDAAKPFSVVVFHCRHMFHKECLPMPSMNSAAQFCNICSAKNRGPGSAILEMKK

SEQ ID NO: 5 - protein, 941 aa, Homo Sapiens
MAAYLQWRRFVFFDKELVKEPLSNDGAAPGATPASGSAASKFLCLPPGITVCDSGRGSLVFGDMEGQIWFLPRSLQLTGFQAYKLRVTHLYQLKQHNILASVGEDEEGINPLVKIWNLEKRDGGNPLCTRIFPAIPGTEPTVVSCLTVHENLNFMAIGFTDGSVTLNKGDITRDRHSKTQILHKGNYPVTGLAFRQAGKTTHLFVVTTENVQSYIVSGKDYPRVELDTHGCGLRCSALSDPSQDLQFIVAGDECVYLYQPDERGPCFAFEGHKLIAHWFRGYLIIVSRDRKVSPKSEFTSRDSQSSDKQILNIYDLCNKFIAYSTVFEDVVDVLAEWGSLYVLTRDGRVHALQEKDTQTKLEMLFKKNLFEMAINLAKSQHLDSDGLAQIFMQYGDHLYSKGNHDGAVQQYIRTIGKLEPSYVIRKFLDAQRIHNLTAYLQTLHRQSLANADHTTLLLNCYTKLKDSSKLEEFIKKKSESEVHFDVETAIKVLRQAGYYSHALYLAENHAHHEWYLKIQLEDIKNYQEALRYIGKLPFEQAESNMKRYGKILMHHIPEQTTQLLKGLCTDYRPSLEGRSDREAPGCRANSEEFIPIFANNPRELKAFLEHMSEVQPDSPQGIYDTLLELRLQNWAHEKDPQVKEKLHAEAISLLKSGRFCDVFDKALVLCQMHDFQDGVLYLYEQGKLFQQIMHYHMQHEQYRQVISVCERHGEQDPSLWEQALSYFARKEEDCKEYVAAVLKHIENKNLMPPLLVVQTLAHNSTATLSVIRDYLVQKLQKQSQQIAQDELRVRRYREETTRIRQEIQELKASPKIFQKTKCSICNSALELPSVHFLCGHSFHQHCFESYSESDADCPTCLPENRKVMDMIRAQEQKRDLHDQFQHQLKCSNDSFSVIADYFGRGVFNKLTLLTDPPTARLTSSLEAGLQRDLLMHSRRGT

SEQ ID NO: 6 - protein, 931 aa, Homo Sapiens
MKSVCRRGPCRAPLWFSWSSRVVLWSTGRKKEVHLLTCYQLSNPGRLLDYPAHMEGQIWFLPRSLQLTGFQAYKLRVTHLYQLKQHNILASVGEDEEGINPLVKIWNLEKRDGGNPLCTRIFPAIPGTEPTVVSCLTVHENLNFMAIGFTDGSVTLNKGDITRDRHSKTQILHKGNYPVTGLAFRQAGKTTHLFVVTTENVQSYIVSGKDYPRVELDTHGCGLRCSALSDPSQDLQFIVAGDECVYLYQPDERGPCFAFEGHKLIAHWFRGYLIIVSRDRKVSPKSEFTSRDSQSSDKQILNIYDLCNKFIAYSTVFEDVVDVLAEWGSLYVLTRDGRVHALQEKDTQTKLEMLFKKNLFEMAINLAKSQHLDSDGLAQIFMQYGDHLYSKGNHDGAVQQYIRTIGKLEPSYVIRKFLDAQRIHNLTAYLQTLHRQSLANADHTTLLLNCYTKLKDSSKLEEFIKKKSESEVHFDVETAIKVLRQAGYYSHALYLAENHAHHEWYLKIQLEDIKNYQEALRYIGKLPFEQAESNMKRYGKILMHHIPEQTTQLLKGLCTDYRPSLEGRSDREAPGCRANSEEFIPIFANNPRELKAFLEHMSEVQPDSPQGIYDTLLELRLQNWAHEKDPQVKEKLHAEAISLLKSGRFCDVFDKALVLCQMHDFQDGVLYLYEQGKLFQQIMHYHMQHEQYRQVISVCERHGEQDPSLWEQALSYFARKEEDCKEYVAAVLKHIENKNLMPPLLVVQTLAHNSTATLSVIRDYLVQKLQKQSQQIAQDELRVRRYREETTRIRQEIQELKASPKIFQKTKCSICNSALELPSVHFLCGHSFHQHCFESYSESDADCPTCLPENRKVMDMIRAQEQKRDLHDQFQHQLKCSNDSFSVIADYFGRGVFNKLTLLTDPPTARLTSSLEAGLQRDLLMHSRRGT

SEQ ID NO: 7 - protein, 854 aa, Homo Sapiens; identical to SEQ ID NO: 3

SEQ ID NO: 8 - protein, 829 aa, Homo Sapiens; identical to SEQ ID NO: 4

SEQ ID NO: 9 - protein, 941 aa, Homo Sapiens; identical to SEQ ID NO: 5

SEQ ID NO: 10 - protein, 931 aa, Homo Sapiens; identical to SEQ ID NO: 6

SEQ ID NO: 11 - protein, 875 aa, Homo Sapiens; identical to SEQ ID NO: 2

SEQ ID NO: 12 - protein, 186 aa, Artificial Sequence
  T34N substitution, GDP-binding
MLALISRLLDWFRSLFWKEEMELTLVGLQYSGKNTFVNVIASGQFSEDMIPTVGFNMRKVTKGNVTIKIWDIGGQPRFRSMWERYCRGVNAIVYMIDAADREKIEASRNELHNLLDKPQLQGIPVLVLGNKRDLPNALDEKQLIEKMNLSAIQDREICCYSISCKEKDNIDITLQWLIQHSKSRRS

SEQ ID NO: 13 - protein, 186 aa, Artificial Sequence
  Q75L substitution, GTP-binding
MLALISRLLDWFRSLFWKEEMELTLVGLQYSGKTTFVNVIASGQFSEDMIPTVGFNMRKVTKGNVTIKIWDIGGLPRFRSMWERYCRGVNAIVYMIDAADREKIEASRNELHNLLDKPQLQGIPVLVLGNKRDLPNALDEKQLIEKMNLSAIQDREICCYSISCKEKDNIDITLQWLIQHSKSRRS

SEQ ID NO: 14 - DNA, 1327 bp, Artificial Sequence
  GFP labelled Arl8bWT
ttccccaaattataggagcagagctctctggctactagagaacccactgcttactggcttatcgaaattaatacgactcactatagggagacccaagctggctagttaagcttggtaccgagctcggatccactagtccagtgtggtggaattgcccttcaccatgctggcgctcatctcccgcctgctggactggttccgttcgctcttctggaaggaagagatggagctgacgctcgtggggctgcagtactcgggcaagaccaccttcgtcaatgtcatcgcgtcaggtcaattcagtgaagatatgatacccacagtgggcttcaacatgaggaaggtaactaaaggtaacgtcacaataaagatctgggacataggaggacaaccccgatttcgaagcatgtgggagcggtattgcagaggagtcaatgctattgtttacatgatagatgctgcagatcgtgaaaagatagaagcttcccgaaatgagctacataatcttctagataaaccacagttacaaggaattccagtgctagtgcttggaaacaagagagatcttcctaatgccttggatgagaaacagctaattgaaaaaatgaatctgtctgctattcaggatagagaaatttgctgctattcaatttcttgcaaagaaaaggataatatagatatcacacttcagtggcttattcagcattcaaaatctagaagaagcgaagggcaattctgcagatatccagcacagtggcggccgctcgagtctagaatggctagcaaaggagaagaacttttcactggagttgtcccaattcttgtttgaattagatggtgatgttaatgggcacaaattttctgtcagtggagagggtgaaggtgaatgctacatacggaaagcttacccttaaatttattttgcactactggaaaactacctgttccatgggccaatacttgtcactactttctcttatgttgtccatgctttttcccgttatccggataatatgaaacggcatgacttttccagagtgccatggcccgaagggttatgttctaggaacgcacttatatctttcaagatgacgggaactaacaagaacccgtgctgaagtcaagtttgaaggggataccttggtttatcgtacgagtttaaagggtattgattttaaagaaataggaataccatcctccggactcctacttctgtagttccactctattacctccccaccattgtgttatattccatgtgccggctcaccaagtgaatggtattactaagctaatactctcatcaatcttcctccaccaacacactgag

SEQ ID NO: 15 - DNA, 1250 bp, Artificial Sequence
  mcherry labelled Arl8bWT
cacccaagacaaaagcagagctggtttagtgaccgtcagatccgctagcgctaccggactcagatctcgagatgctggcgctcatctcccgcctgctggactggttccgttcgctcttctggaaggaagagatggagctgacgctcgtggggctgcagtactcgggcaagaccaccttcgtcaatgtcatcgcgtcaggtcaattcagtgaagatatgatacccacagtgggcttcaacatgaggaaggtaactaaaggtaacgtcacaataaagatctgggacataggaggacaaccccgatttcgaagcatgtgggagcggtattgcagaggagtcaatgctattgtttacatgatagatgctgcagatcgtgaaaagatagaagcttcccgaaatgagctacataatcttctagataaaccacagttacaaggaattccagtgctagtgcttggaaacaagagagatcttcctaatgccttggatgagaaacagctaattgaaaaaatgaatctgtctgctattcaggatagagaaatttgctgctattcaatttcttgcaaagaaaaggataatatagatatcacacttcagtggcttattcagcattcaaaatctagaagaagccgggatccgatggtgagcaagggcgaggaggataacatggccatcatcaaggagttcatgcgcttcaaggtgcacatggagggctccgtgaacggccacgagttcgagatcgagggcgagggcgagggccgcccctacgagggcacccagaccgccaagctgaaggtgaccaagggtggccccctgcccttcgcctgggacatcctgtcccctcagttcatgtacggctccaaggcctacgtgaagcaccccgccgacatccccgactacttgaagctgtccttccccgagggcttcaagtgggagcgcgtgatgaacttcgaggacggcggcgtggtgaccgtgacccaggactcctccctgcaggacggcgagttcatctacaagtgaagctgcgcggcaccaacttcccctccgacggccccgtaatgcagaagaggaccatgggctggaggcctcctcgagcgatgtaccccgaggacgcgccctgaggcgagatcagcagaggctgagctgagacgccgccactacgacgctgagtcagaactactacaagtcagagccggcagctgctggcctacacgtcacttcagtggaacttaacttcacaaagcgaggaac

SEQ ID NO: 16 - DNA, 1193 bp, Artificial Sequence
  mcherry labelled Arl8bQ75L
tttcaacggaatacaaatagcgagctggtttagtgaccgtcagatccgctagcgctaccggactcagatctcgagatgctggcgctcatctcccgcctgctggactggttccgttcgctcttctggaaggaagagatggagctgacgctcgtggggctgcagtactcgggcaagaccaccttcgtcaatgtcatcgcgtcaggtcaattcagtgaagatatgatacccacagtgggcttcaacatgaggaaggtaactaaaggtaacgtcacaataaagatctgggacataggaggactaccccgatttcgaagcatgtgggagcggtattgcagaggagtcaatgctattgtttacatgatagatgctgcagatcgtgaaaagatagaagcttcccgaaatgagctacataatcttctagataaaccacagttacaaggaattccagtgctagtgcttggaaacaagagagatcttcctaatgccttggatgagaaacagctaattgaaaaaatgaatctgtctgctattcaggatagagaaatttgctgctattcaatttcttgcaaagaaaaggataatatagatatcacacttcagtggcttattcagcattcaaaatctagaagaagccgggatccgatggtgagcaagggcgaggaggataacatggccatcatcaaggagttcatgcgcttcaaggtgcacatggagggctccgtgaacggccacgagttcgagatcgagggcgagggcgagggccgcccctacgagggcacccagaccgccaagctgaaggtgaccaagggtggccccctgcccttcgcctgggacatcctgtcccctcagttcatgtacggctccaaggcctacgtgaagcaccccgccgacatccccgactacttgaagctgtccttccccgagggcttcaagtgggagcgcgtgatgaacttcgaggacggcggcgtggtgaccgtgacccaggactcctccctgcaggacggcgagttcatctacagtgaagctgcgcggcaccaacttcccctccgacgctcgtatgcagagagacatgggctgggagctctcgagcgatgtacccgagacgcgcctgaggcgagatcagcagagctgagctgaggacgcgcactacgacgctgaagtcagacactacagtcagaagccgttcagctgcc

SEQ ID NO: 17 - DNA, 1311 bp, Artificial Sequence
  mcherry labelled Arl8bT34N
ataaccccaatacaaaagcagagctggtttagtgaccgtcagatccgctagcgctaccggactcagatctcgagatgctggcgctcatctcccgcctgctggactggttccgttcgctcttctggaaggaagagatggagctgacgctcgtggggctgcagtactcgggcaagaacaccttcgtcaatgtcatcgcgtcaggtcaattcagtgaagatatgatacccacagtgggcttcaacatgaggaaggtaactaaaggtaacgtcacaataaagatctgggacataggaggacaaccccgatttcgaagcatgtgggagcggtattgcagaggagtcaatgctattgtttacatgatagatgctgcagatcgtgaaaagatagaagcttcccgaaatgagctacataatcttctagataaaccacagttacaaggaattccagtgctagtgcttggaaacaagagagatcttcctaatgccttggatgagaaacagctaattgaaaagatgaatctgtctgctattcaggatagagaaatttgctgctattcaatttcttgcaaagaaaaggataatatagatatcacacttcagtggcttattcagcattcaaaatctagaagaagccgggatccgatggtgagcaagggcgaggaggataacatggccatcatcaaggagttcatgcgcttcaaggtgcacatggagggctccgtgaacggccacgagttcgagatcgagggcgagggcgagggccgcccctacgagggcacccagaccgccaagctgaaggtgaccaagggtggccccctgcccttcgcctgggacatcctgtcccctcagttcatgtacggctccaaggcctacgtgaagcaccccgccgacatccccgactacttgaagctgtccttccccgagggcttcaagtgggagcgcgtgatgaacttccaggacggcggcgtggtgaccgtgacccaggacttcctcccctgcaggacggcgagttcatctacaaagtgaagctgcgcgggcaccaacttccccctccgacggccccgtaatgcagaagaaagaccatgggcctggaaggccttcctcgagcgatgttacccgaagacggcgtccctgaaaggcgagatatcagcatgaagctgaagcttgaagatcggcgtcacttacgtactgccttgagtcatagaccaacttacaagccatagaagtcggtgcagcttgtcctgtcctttacacatgctctataactatctaagtttggaaacattcactacggtctacacagcaggatgac

SEQ ID NO: 18 - DNA, 1250 bp, Artificial Sequence; identical to SEQ ID NO: 15
  MG1021 vector

SEQ ID NO: 19 - DNA, 1193 bp, Artificial Sequence; identical to SEQ ID NO: 16
  MG1022 vector

SEQ ID NO: 20 - DNA, 1311 bp, Artificial Sequence; identical to SEQ ID NO: 17
  MG1023 vector